European Patent Specification EP 3 215 168 B1, published August 2, 2023. Title: ALTERING GENE EXPRESSION IN MODIFIED T CELLS AND USES THEREOF. Applicant: The Trustees of the University of Pennsylvania Zhao, Yangbing Ren, Jiangtao Liu, Xiaojun June, Carl H. The sequence listing filed with the application follows.

SEQUENCE LISTING (13 sequences)

SEQ ID NO: 1 - DNA, 20 bp, Artificial Sequence
  Synthetic sequence
tgtgctagacatgaggtcta

SEQ ID NO: 2 - DNA, 20 bp, Artificial Sequence
  Synthetic sequence
gcagtatctggagtcattga

SEQ ID NO: 3 - DNA, 20 bp, Artificial Sequence
  Synthetic sequence
cgcgagcacagctaaggcca

SEQ ID NO: 4 - DNA, 20 bp, Artificial Sequence
  Synthetic sequence
ggcgccctggccagtcgtct

SEQ ID NO: 5 - DNA, 20 bp, Artificial Sequence
  Synthetic sequence
gagggtccagatgcccagca

SEQ ID NO: 6 - DNA, 24 bp, Artificial Sequence
  Synthetic sequence
tcatgtcctaaccctgatcctctt

SEQ ID NO: 7 - DNA, 23 bp, Artificial Sequence
  Synthetic sequence
ttggacttttcccagctgacaga

SEQ ID NO: 8 - DNA, 24 bp, Artificial Sequence
  Synthetic sequence
taccaggaccagacagctcttaga

SEQ ID NO: 9 - DNA, 24 bp, Artificial Sequence
  Synthetic sequence
tctcacctaatctcctccaggcat

SEQ ID NO: 10 - RNA, 54 nt, Artificial Sequence
  Synthetic sequence
rargrgrargrgrarururcrgrgrararcrcrcrararurcrarcrurgrarc

SEQ ID NO: 11 - DNA, 48 bp, Artificial Sequence
  Synthetic sequence
rcrargrurgrarururgrgrgrururcrcrgrararurcrcrurcct

SEQ ID NO: 12 - DNA, 54 bp, Artificial Sequence
  Synthetic sequence
rarcrcrurcrcrururcrcrcrarururcrarcrcrcrarcrcrargrcrurc

SEQ ID NO: 13 - DNA, 48 bp, Artificial Sequence
  Synthetic sequence
rgrcrurgrgrurgrgrgrurgrararurgrgrgrarargrgrarggt